European Patent Application EP 4 299 593 A1, published January 3, 2024. Title: CLDN18.2 ANTIGEN-BINDING PROTEIN AND USE THEREOF. Applicant: Oricell Therapeutics Co.,Ltd. The sequence listing filed with the application follows.

SEQUENCE LISTING (93 sequences)

SEQ ID NO: 1 - protein, 118 aa, Artificial Sequence
  5E6 VH
EVQLQQSGPELVKPGASVKMSCKASGYTFTNYVMNWVKQKPGQGLEWIGYINPYNDGTKYNERFKGKATLTSDKSSSTAFMEVSSLTSEDSAVYYCARLYRGNAMDYWGQGTSVTVSS

SEQ ID NO: 2 - protein, 5 aa, Artificial Sequence
  5E6 HCDR1
NYVMN

SEQ ID NO: 3 - protein, 17 aa, Artificial Sequence
  5E6 HCDR2
YINPYNDGTKYNERFKG

SEQ ID NO: 4 - protein, 9 aa, Artificial Sequence
  5E6 HCDR3
LYRGNAMDY

SEQ ID NO: 5 - protein, 114 aa, Artificial Sequence
  5E6VL 7E3 VL
DIVMTQSPSSLTVTVREKVTLSCKSSQSLLNSGNQKNYLTWYQQKPGQPPKLLIYWASTRESGVPDRFTGSGSGTDFTLTISSVQAEDLAVYYCQNVYIYPFTFGAGTKLELKR

SEQ ID NO: 6 - protein, 17 aa, Artificial Sequence
  5E6LCDR1 3A6LCDR1 7E3LCDR1 17B10LCDR1 IMAB362LCDR1
KSSQSLLNSGNQKNYLT

SEQ ID NO: 7 - protein, 7 aa, Artificial Sequence
  5E6LCDR2 3A6LCDR2 7E3LCDR2 17B10LCDR2 IMAB362LCDR2
WASTRES

SEQ ID NO: 8 - protein, 9 aa, Artificial Sequence
  5E6LCDR3 7E3LCDR3
QNVYIYPFT

SEQ ID NO: 9 - protein, 118 aa, Artificial Sequence
  3A6 VH
EVQLVESGGDLVQPGGSLKLSCAASGFTLSRYGMSWVRQTPDKRLEWVSTIISGGINTYYSDSVKGRFSISRDNARNTLYLQMSSLKSEDTAMYYCGRLYYGNAMDYWGQGTAVTVSS

SEQ ID NO: 10 - protein, 5 aa, Artificial Sequence
  3A6 HCDR1
RYGMS

SEQ ID NO: 11 - protein, 17 aa, Artificial Sequence
  3A6 HCDR2
TIISGGINTYYSDSVKG

SEQ ID NO: 12 - protein, 9 aa, Artificial Sequence
  3A6 HCDR3
LYYGNAMDY

SEQ ID NO: 13 - protein, 114 aa, Artificial Sequence
  3A6 VL
DIVMTQSPSSLTVTAGEKVTMSCKSSQSLLNSGNQKNYLTWYQQKPGQPPKLLIYWASTRESGVPDRFTGSGSGTHFTLTISSVQAEDLAVYYCQNDYSYPLTFGAGTKLELKR

SEQ ID NO: 14 - protein, 9 aa, Artificial Sequence
  3A6 LCDR3
QNDYSYPLT

SEQ ID NO: 15 - protein, 118 aa, Artificial Sequence
  7E3 VH
EVQLQQSGPELVKPGASVKMSCKASGYTFTNYIIHWVKQKPGQGLEWIGYINPYTDGPKYNEKFKGRATLTSDKSSSTAYMEFSSLTSEDSAVYYCARLNRGNAMDYWGQGTSVTVSS

SEQ ID NO: 16 - protein, 5 aa, Artificial Sequence
  7E3HCDR1 14E12HCDR1 17B10HCDR1
NYIIH

SEQ ID NO: 17 - protein, 17 aa, Artificial Sequence
  7E3HCDR2 14E12HCDR2 17B10HCDR2
YINPYTDGPKYNEKFKG

SEQ ID NO: 18 - protein, 9 aa, Artificial Sequence
  7E3HCDR3 14E12HCDR3 17B10HCDR3
LNRGNAMDY

SEQ ID NO: 19 - protein, 118 aa, Artificial Sequence
  14E12VH 17B10VH
EVQLQESGPELVKPGASVKMSCKASGYTFTNYIIHWVKQKPGQGLEWIGYINPYTDGPKYNEKFKGRATLTSDKSSSTAYMEFSSLTSEDSAVYYCARLNRGNAMDYWGQGTSVTVSS

SEQ ID NO: 20 - protein, 114 aa, Artificial Sequence
  14E12 VL
DIVMTQSPSSLSVSAGEKVTMSCKSSQSLLNNGNQKNYLAWYQQKPGQPPKLLIYGASTRESGVPDRFTGSGSGTDFALTISSVQAEDLAVYYCQNDLYYPFTFGSGTKLDIKR

SEQ ID NO: 21 - protein, 17 aa, Artificial Sequence
  14E12 LCDR1
KSSQSLLNNGNQKNYLA

SEQ ID NO: 22 - protein, 7 aa, Artificial Sequence
  14E12 LCDR2
GASTRES

SEQ ID NO: 23 - protein, 9 aa, Artificial Sequence
  14E12 LCDR3
QNDLYYPFT

SEQ ID NO: 24 - protein, 114 aa, Artificial Sequence
  17B10 VL
DIVMTQSPSSLTVTAGEKVTMNCKSSQSLLNSGNQKNYLTWYQQKPGQPPKLLIYWASTRESGVPDRFTGSGSGTDFTLTISSVQAEDLAVYYCQNDYSFPFTFGSGTKLEIKR

SEQ ID NO: 25 - protein, 9 aa, Artificial Sequence
  17B10 LCDR3
QNDYSFPFT

SEQ ID NO: 26 - DNA, 354 bp, Artificial Sequence
  5E6 VH DNA
gaggtccagctgcagcagtctggacctgagctggtaaagcctggggcttcagtgaagatgtcctgcaaggcttctggatacacattcactaactatgttatgaactgggtgaagcagaagcctgggcagggccttgagtggattggatatattaatccttacaatgatggtactaagtacaatgagaggttcaaaggcaaggccacactgacttcagacaaatcctccagcacagccttcatggaggtcagcagcctgacctctgaggactctgcggtctactactgtgcaagactatatagaggcaatgctatggactactggggtcaaggaacctcggtcaccgtctcctca

SEQ ID NO: 27 - DNA, 342 bp, Artificial Sequence
  5E6VL DNA 7E3 VL DNA
gacattgtgatgacacagtctccatcctccctgactgtgacagtaagagagaaggtcactttgagctgcaagtccagtcagagtctgttaaacagtggaaatcaaaagaactacttgacctggtaccagcagaaaccagggcagcctcctaaacttttgatctactgggcatccactagggaatctggggtccctgatcgcttcacaggcagtggatctggcacagatttcactctcaccatcagcagtgtgcaggctgaagacctggcagtttattactgtcagaatgtttatatttatccgttcacgttcggtgctgggaccaagctggagctgaaacgg

SEQ ID NO: 28 - DNA, 354 bp, Artificial Sequence
  3A6 VH DNA
gaggtgcagttggtggagtctgggggagacttagtgcagcctggagggtccctgaaactctcctgtgcagcctctggattcactttaagtcgttatggcatgtcttgggttcgccagactcctgacaagaggctggagtgggtctcaaccattattagtggtggtattaacacctactattcagacagtgtgaaggggcgattctccatctccagagacaatgccaggaacaccctgtacctgcaaatgagcagtctgaagtctgaggacacagccatgtattactgtggaagactctactatggcaatgctatggactactgggggcaaggaaccgctgtcaccgtctcctca

SEQ ID NO: 29 - DNA, 342 bp, Artificial Sequence
  3A6 VL DNA
gacattgtgatgacacagtctccatcctccctgactgtgacagcaggagagaaggtcactatgagctgcaagtccagtcagagtctgttaaacagtggaaatcaaaagaactacttgacctggtaccagcagaaaccagggcagcctcctaaactgttgatctactgggcatccactagggaatctggggtccctgatcgcttcacaggcagtggatctggaacacatttcactctcaccatcagcagtgtgcaggctgaagacctggcagtttattactgtcagaatgattatagttatcctctcacgttcggtgctgggaccaagctggagctgaaacgg

SEQ ID NO: 30 - DNA, 354 bp, Artificial Sequence
  7E3 VH DNA
gaggtccagttgcagcagtctggacctgagctggtaaagcctggggcttcagtgaagatgtcctgcaaggcttctggatacacattcactaactatattatacactgggtgaagcagaagcctgggcagggccttgagtggattggatatattaatccttacactgatggtcctaagtacaatgagaagttcaaaggcagggccacactgacttcagacaaatcctccagtacagcctacatggagttcagcagcctgacctctgaggactctgcggtctattactgtgcaagactaaatagaggcaatgctatggactactggggtcaaggaacctcagtcaccgtctcctca

SEQ ID NO: 31 - DNA, 354 bp, Artificial Sequence
  14E12 VH DNA  17B10 VH DNA
gaggtgcagctgcaggagtctggacctgagctggtaaagcctggggcttcagtgaagatgtcctgcaaggcttctggatacacattcactaactatattatacactgggtgaagcagaagcctgggcagggccttgagtggattggatatattaatccttacactgatggtcctaagtacaatgagaagttcaaaggcagggccacactgacttcagacaaatcctccagtacagcctacatggagttcagcagcctgacctctgaggactctgcggtctattactgtgcaagactaaatagaggcaatgctatggactactggggtcaaggaacctcagtcaccgtctcctca

SEQ ID NO: 32 - DNA, 342 bp, Artificial Sequence
  14E12 VL DNA
gatattgtgatgacccagtctccatcttccctgagtgtgtcagcaggagagaaggtcactatgagctgcaagtccagtcagagtctgttaaacaatggaaatcaaaagaactatttggcctggtaccagcagaaaccagggcagcctcctaaactgttgatctacggggcatccactagggaatctggggtccctgatcgcttcacaggcagtggatctggaaccgatttcgctcttaccatcagcagtgtgcaggctgaagacctggcagtttattactgtcagaatgatctttattatccattcacgttcggctcggggacaaagttggacataaaacgg

SEQ ID NO: 33 - DNA, 342 bp, Artificial Sequence
  17B10 VL DNA
gatattgtgatgacccagtctccatcctccctgactgtgacagcaggagagaaggtcactatgaactgcaagtccagtcagagtctgttaaacagtggaaatcaaaagaactacttgacctggtaccagcagaaaccagggcagcctcctaaactgttgatctactgggcatccactagggaatctggggtccctgatcggttcacaggcagtggatctggaacagatttcactctcaccatcagcagtgtgcaggctgaagacctggcagtttattactgtcagaatgattatagttttccattcacgttcggctcggggacaaagttggaaataaaacgg

SEQ ID NO: 34 - protein, 30 aa, Artificial Sequence
  5E6 H-FR1 7E3 H-FR1
EVQLQQSGPELVKPGASVKMSCKASGYTFT

SEQ ID NO: 35 - protein, 14 aa, Artificial Sequence
  5E6H-FR2 7E3H-FR2 14E12H-FR2 17B10H-FR2
WVKQKPGQGLEWIG

SEQ ID NO: 36 - protein, 32 aa, Artificial Sequence
  5E6 H-FR3
KATLTSDKSSSTAFMEVSSLTSEDSAVYYCAR

SEQ ID NO: 37 - protein, 11 aa, Artificial Sequence
  5E6H-FR4 7E3H-FR4 14E12H-FR4 17B10H-FR4
WGQGTSVTVSS

SEQ ID NO: 38 - protein, 23 aa, Artificial Sequence
  5E6L-FR1 7E3L-FR1
DIVMTQSPSSLTVTVREKVTLSC

SEQ ID NO: 39 - protein, 15 aa, Artificial Sequence
  5E6L-FR2 7E3L-FR2 3A6L-FR2 14E12L-FR2 17B10L-FR2
WYQQKPGQPPKLLIY

SEQ ID NO: 40 - protein, 32 aa, Artificial Sequence
  5E6L-FR3 7E3L-FR3 17B10L-FR3
GVPDRFTGSGSGTDFTLTISSVQAEDLAVYYC

SEQ ID NO: 41 - protein, 11 aa, Artificial Sequence
  5E6L-FR4 7E3L-FR4 3A6L-FR4
FGAGTKLELKR

SEQ ID NO: 42 - protein, 32 aa, Artificial Sequence
  7E3H-FR3 14E12H-FR3 17B10H-FR3
RATLTSDKSSSTAYMEFSSLTSEDSAVYYCAR

SEQ ID NO: 43 - protein, 30 aa, Artificial Sequence
  3A6 H-FR1
EVQLVESGGDLVQPGGSLKLSCAASGFTLS

SEQ ID NO: 44 - protein, 14 aa, Artificial Sequence
  3A6 H-FR2
WVRQTPDKRLEWVS

SEQ ID NO: 45 - protein, 32 aa, Artificial Sequence
  3A6 H-FR3
RFSISRDNARNTLYLQMSSLKSEDTAMYYCGR

SEQ ID NO: 46 - protein, 11 aa, Artificial Sequence
  3A6 H-FR4
WGQGTAVTVSS

SEQ ID NO: 47 - protein, 23 aa, Artificial Sequence
  3A6 L-FR1
DIVMTQSPSSLTVTAGEKVTMSC

SEQ ID NO: 48 - protein, 32 aa, Artificial Sequence
  3A6 L-FR3
GVPDRFTGSGSGTHFTLTISSVQAEDLAVYYC

SEQ ID NO: 49 - protein, 30 aa, Artificial Sequence
  14E12H-FR1 17B10H-FR1
EVQLQESGPELVKPGASVKMSCKASGYTFT

SEQ ID NO: 50 - protein, 23 aa, Artificial Sequence
  14E12 L-FR1
DIVMTQSPSSLSVSAGEKVTMSC

SEQ ID NO: 51 - protein, 32 aa, Artificial Sequence
  14E12 L-FR3
GVPDRFTGSGSGTDFALTISSVQAEDLAVYYC

SEQ ID NO: 52 - protein, 11 aa, Artificial Sequence
  14E12 L-FR4
FGSGTKLDIKR

SEQ ID NO: 53 - protein, 23 aa, Artificial Sequence
  17B10 L-FR1
DIVMTQSPSSLTVTAGEKVTMNC

SEQ ID NO: 54 - protein, 11 aa, Artificial Sequence
  17B10 L-FR4
FGSGTKLEIKR

SEQ ID NO: 55 - protein, 118 aa, Artificial Sequence
  IMAB362 VH
QVQLQQPGAELVRPGASVKLSCKASGYTFTSYWINWVKQRPGQGLEWIGNIYPSDSYTNYNQKFKDKATLTVDKSSSTAYMQLSSPTSEDSAVYYCTRSWRGNSFDYWGQGTTLTVSS

SEQ ID NO: 56 - protein, 114 aa, Artificial Sequence
  IMAB362 VL
DIVMTQSPSSLTVTAGEKVTMSCKSSQSLLNSGNQKNYLTWYQQKPGQPPKLLIYWASTRESGVPDRFTGSGSGTDFTLTISSVQAEDLAVYYCQNDYSYPFTFGSGTKLEIKR

SEQ ID NO: 57 - protein, 5 aa, Artificial Sequence
  IMAB362 HCDR1
SYWIN

SEQ ID NO: 58 - protein, 17 aa, Artificial Sequence
  IMAB362 HCDR2
NIYPSDSYTNYNQKFKD

SEQ ID NO: 59 - protein, 9 aa, Artificial Sequence
  IMAB362 HCDR3
SWRGNSFDY

SEQ ID NO: 60 - protein, 9 aa, Artificial Sequence
  IMAB362 LCDR3
QNDYSYPFT

SEQ ID NO: 61 - DNA, 783 bp, Artificial Sequence
  human CLDN18.1
atgtccaccaccacatgccaagtggtggcgttcctcctgtccatcctggggctggccggctgcatcgcggccaccgggatggacatgtggagcacccaggacctgtacgacaaccccgtcacctccgtgttccagtacgaagggctctggaggagctgcgtgaggcagagttcaggcttcaccgaatgcaggccctatttcaccatcctgggacttccagccatgctgcaggcagtgcgagccctgatgatcgtaggcatcgtcctgggtgccattggcctcctggtatccatctttgccctgaaatgcatccgcattggcagcatggaggactctgccaaagccaacatgacactgacctccgggatcatgttcattgtctcaggtctttgtgcaattgctggagtgtctgtgtttgccaacatgctggtgactaacttctggatgtccacagctaacatgtacaccggcatgggtgggatggtgcagactgttcagaccaggtacacatttggtgcggctctgttcgtgggctgggtcgctggaggcctcacactaattgggggtgtgatgatgtgcatcgcctgccggggcctggcaccagaagaaaccaactacaaagccgtttcttatcatgcctcaggccacagtgttgcctacaagcctggaggcttcaaggccagcactggctttgggtccaacaccaaaaacaagaagatatacgatggaggtgcccgcacagaggacgaggtacaatcttatccttccaagcacgactatgtg

SEQ ID NO: 62 - DNA, 783 bp, Artificial Sequence
  human CLDN18.2
atggccgtgactgcctgtcagggcttggggttcgtggtttcactgattgggattgcgggcatcattgctgccacctgcatggaccagtggagcacccaagacttgtacaacaaccccgtaacagctgttttcaactaccaggggctgtggcgctcctgtgtccgagagagctctggcttcaccgagtgccggggctacttcaccctgctggggctgccagccatgctgcaggcagtgcgagccctgatgatcgtaggcatcgtcctgggtgccattggcctcctggtatccatctttgccctgaaatgcatccgcattggcagcatggaggactctgccaaagccaacatgacactgacctccgggatcatgttcattgtctcaggtctttgtgcaattgctggagtgtctgtgtttgccaacatgctggtgactaacttctggatgtccacagctaacatgtacaccggcatgggtgggatggtgcagactgttcagaccaggtacacatttggtgcggctctgttcgtgggctgggtcgctggaggcctcacactaattgggggtgtgatgatgtgcatcgcctgccggggcctggcaccagaagaaaccaactacaaagccgtttcttatcatgcctcaggccacagtgttgcctacaagcctggaggcttcaaggccagcactggctttgggtccaacaccaaaaacaagaagatatacgatggaggtgcccgcacagaggacgaggtacaatcttatccttccaagcacgactatgtg

SEQ ID NO: 63 - DNA, 792 bp, Artificial Sequence
  mouse CLDN18.1
atggccaccaccacgtgccaggtggtagggcttctcctgtccctcctgggtctggccggctgcatagccgccactgggatggacatgtggagcactcaagacctgtatgacaacccagtcaccgccgtgttccagtatgaagggctctggaggagttgcgtgcaacagagctcggggttcaccgagtgccggccatacttcaccatcctgggccttccagccatgctgcaagctgtacgagccctgatgatcgtgggcattgttctgggggtcatcggtatcctcgtgtccatcttcgccctgaagtgcattcgcattggtagcatggatgactctgccaaggccaagatgactctgacttctgggatcttgttcatcatctccggcatctgtgcaatcattggtgtgtctgtgtttgccaacatgctggtgaccaacttctggatgtccacagctaacatgtacagcggcatgggcggcatgggtggcatggtgcagaccgttcagaccaggtacacctttggtgcagctctgttcgtgggctgggttgctggaggcctcaccctgattgggggagtgatgatgtgcatcgcctgccgtggcctgacaccagatgacagcaacttcaaagctgtgtcttaccatgcctctggccaaaatgttgcctacaggcctggaggctttaaggccagcactggctttgggtccaacaccagaaacaagaagatctacgatgggggtgcccgcacagaagacgatgaacagtctcatcctaccaagtatgactatgtg

SEQ ID NO: 64 - DNA, 792 bp, Artificial Sequence
  mouse CLDN18.2
atgtcggtgaccgcctgccagggcttggggtttgtggtgtcactgatcgggtttgcgggcatcattgcagccacttgtatggaccagtggagcacccaggatttatacaacaacccggtgaccgctgtattcaactaccaagggctatggcgttcatgcgtccgagagagctctggcttcaccgagtgccgaggctacttcaccctgttggggttgccagccatgctgcaagctgtacgagccctgatgatcgtgggcattgttctgggggtcatcggtatcctcgtgtccatcttcgccctgaagtgcattcgcattggtagcatggatgactctgccaaggccaagatgactctgacttctgggatcttgttcatcatctccggcatctgtgcaatcattggtgtgtctgtgtttgccaacatgctggtgaccaacttctggatgtccacagctaacatgtacagcggcatgggcggcatgggtggcatggtgcagaccgttcagaccaggtacacctttggtgcagctctgttcgtgggctgggttgctggaggcctcaccctgattgggggagtgatgatgtgcatcgcctgccgtggcctgacaccagatgacagcaacttcaaagctgtgtcttaccatgcctctggccaaaatgttgcctacaggcctggaggctttaaggccagcactggctttgggtccaacaccagaaacaagaagatctacgatgggggtgcccgcacagaagacgatgaacagtctcatcctaccaagtatgactatgtg

SEQ ID NO: 65 - DNA, 783 bp, Artificial Sequence
  cynomolgus monkey CLDN18.1
atgtccaccaccacatgccaagtggtggcgttcctcctgtccatcctggggctggcgggctgcatcgcggccaccgggatggacatgtggagcacccaggacctgtacgacaaccccgtcacctctgtgttccagtacgaagggctgtggaggagctgcgtgaggcagagctcggggttcaccgagtgcaggccctatttcaccatcctgggccttccagccatgctgcaggcagtgcgagccctgatgatcgtaggcatcgtcctgggtgccattggcctcctggtatccatctttgccctgaaatgcatccgcattggcagcatggaggactctgccaaagccaacatgacactgacctccgggatcatgttcattgtctcaggtctttgtgcaattgctggagtgtctgtgtttgccaacatgctggtgactaacttctggatgtccacagctaacatgtacaccggcatgggtgggatggtgcagactgttcagaccaggtacacatttggtgcagctctgttcgtgggctgggtcgctggaggcctcacactaattgggggtgtgatgatgtgcatcgcctgccggggcctggcaccagaagaaaccaactacaaagccgtttcttatcatgcctcgggccacagtgttgcctacaagcctggaggcttcaaggccagcactggctttgggtccaacaccaaaaacaagaagacatatgatgggggtgcccacacagaggacgagttacaatcttatccttccaagcacgactatgtg

SEQ ID NO: 66 - DNA, 783 bp, Artificial Sequence
  cynomolgus monkey CLDN18.2
atggccgtgactgcctgtcagggcttggggttcgtggtttcactgattgggattgcgggcatcattgctgccacctgcatggaccagtggagcacccaagacttgtacaacaaccccgtgacagctgtattcaactaccaggggctgtggcgctcctgtgtccgagagagctctggcttcaccgagtgcaggggctacttcaccctgctggggctgccagccatgctgcaggcagtgcgagccctgatgatcgtaggcatcgtcctgggtgccattggcctcctggtatccatctttgccctgaaatgcatccgcattggcagcatggaggactctgccaaagccaacatgacactgacctccgggatcatgttcattgtctcaggtctttgtgcaattgctggagtgtctgtgtttgccaacatgctggtgactaacttctggatgtccacagctaacatgtacaccggcatgggtgggatggtgcagactgttcagaccaggtacacatttggtgcggctctgttcgtgggctgggtcgctggaggcctcacactaattgggggtgtgatgatgtgcatcgcctgccggggcctggcaccagaagaaaccaactacaaagccgtttcttatcatgcctcgggccacagtgttgcctacaagcctggaggcttcaaggccagcactggctttgggtccaacaccaaaaacaagaagacatatgatgggggtgcccacacagaggacgagttacaatcttatccgtccaagcacgactatgtg

SEQ ID NO: 67 - protein, 9 aa, Artificial Sequence
  5E6HCDR3  3A6HCDR3  7E3HCDR3 14E12HCDR3 17B10 HCDR3
  misc_feature (2)..(2): Xaa = Asn or Tyr
  misc_feature (3)..(3): Xaa = Arg or Tyr
LXXGNAMDY

SEQ ID NO: 68 - protein, 17 aa, Artificial Sequence
  5E6 HCDR2 7E3HCDR2 14E12HCDR2 17B10 HCDR2
  misc_feature (6)..(6): Xaa = Asn or Thr
  misc_feature (9)..(9): Xaa = Pro or Thr
  misc_feature (14)..(14): Xaa = Lys or Arg
YINPYXDGXKYNEXFKG

SEQ ID NO: 69 - protein, 9 aa, Artificial Sequence
  5E6LCDR3 7E3LCDR3 14E12LCDR3 3A6LCDR3 17B10LCDR3
  misc_feature (3)..(3): Xaa = Asp or Val
  misc_feature (4)..(4): Xaa = Leu or Tyr
  misc_feature (5)..(5): Xaa = Ile  Ser or Tyr
  misc_feature (6)..(6): Xaa = Phe or Tyr
  misc_feature (8)..(8): Xaa = Phe or Leu
QNXXXXPXT

SEQ ID NO: 70 - protein, 7 aa, Artificial Sequence
  5E6LCDR3 3A6LCDR3 7E3LCDR3 17B10LCDR3 IMAB362LCDR2 14E12LCDR2
  misc_feature (1)..(1): Xaa = Gly or Trp
XASTRES

SEQ ID NO: 71 - protein, 17 aa, Artificial Sequence
  5E6LCDR1 3A6LCDR1 7E3LCDR1 17B10LCDR1 IMAB362LCDR1  14E12LCDR1
  misc_feature (9)..(9): Xaa = Asn or Ser
  misc_feature (17)..(17): Xaa = Ala or Thr
KSSQSLLNXGNQKNYLX

SEQ ID NO: 72 - protein, 30 aa, Artificial Sequence
  5E6H-FR1 7E3H-FR1 3A6H-FR1 14E12H-FR1 17B10H-FR1
  misc_feature (5)..(5): Xaa = Gln or Val
  misc_feature (6)..(6): Xaa = Glu or Gln
  misc_feature (9)..(9): Xaa = Gly or Pro
  misc_feature (10)..(10): Xaa = Asp or Glu
  misc_feature (13)..(13): Xaa = Lys or Gln
  misc_feature (16)..(16): Xaa = Ala or Gly
  misc_feature (18)..(18): Xaa = Leu or Val
  misc_feature (20)..(20): Xaa = Leu or Met
  misc_feature (23)..(23): Xaa = Ala or Lys
  misc_feature (27)..(27): Xaa = Phe or Tyr
  misc_feature (29)..(29): Xaa = Phe or Leu
  misc_feature (30)..(30): Xaa = Ser or Thr
EVQLXXSGXXLVXPGXSXKXSCXASGXTXX

SEQ ID NO: 73 - protein, 14 aa, Artificial Sequence
  5E6H-FR2 7E3H-FR2 14E12H-FR2 17B10H-FR2 3A6H-FR2
  misc_feature (3)..(3): Xaa = Lys or Arg
  misc_feature (5)..(5): Xaa = Lys or Thr
  misc_feature (7)..(7): Xaa = Asp or Gly
  misc_feature (8)..(8): Xaa = Lys or Gln
  misc_feature (9)..(9): Xaa = Gly or Arg
  misc_feature (13)..(13): Xaa = Ile or Val
  misc_feature (14)..(14): Xaa = Gly or Ser
WVXQXPXXXLEWXX

SEQ ID NO: 74 - protein, 11 aa, Artificial Sequence
  5E6H-FR2 7E3H-FR2 14E12H-FR2 17B10H-FR4 3A6 H-FR4
  misc_feature (6)..(6): Xaa = Ala or Ser
WGQGTXVTVSS

SEQ ID NO: 75 - protein, 23 aa, Artificial Sequence
  5E6L-FR1 7E3L-FR1 3A6L-FR1 14E12L-FR1 17B10 L-FR1
  misc_feature (12)..(12): Xaa = Ser or Thr
  misc_feature (14)..(14): Xaa = Ser or Thr
  misc_feature (15)..(15): Xaa = Ala or Val
  misc_feature (16)..(16): Xaa = Gly or Arg
  misc_feature (21)..(21): Xaa = Leu or Met
  misc_feature (22)..(22): Xaa = Asn or Ser
DIVMTQSPSSLXVXXXEKVTXXC

SEQ ID NO: 76 - protein, 32 aa, Artificial Sequence
  5E6L-FR3 7E3L-FR3 17B10L-FR3 3A6L-FR3 14E12L-FR3
  misc_feature (14)..(14): Xaa = Asp or His
  misc_feature (16)..(16): Xaa = Ala or Thr
GVPDRFTGSGSGTXFXLTISSVQAEDLAVYYC

SEQ ID NO: 77 - protein, 11 aa, Artificial Sequence
  5E6L-FR4 7E3L-FR4 3A6L-FR4 14E12L-FR4 17B10L-FR4
  misc_feature (3)..(3): Xaa = Ala or Ser
  misc_feature (8)..(8): Xaa = Asp or Glu
  misc_feature (9)..(9): Xaa = Ile or Leu
FGXGTKLXXKR

SEQ ID NO: 78 - protein, 118 aa, Artificial Sequence
  5E6 VH PRT  3A6 VH PRT  7E3 VH PRT  14E12VH PRT17B10 VH PRT
  misc_feature (5)..(5): Xaa = Gln or Val
  misc_feature (6)..(6): Xaa = Glu or Gln
  misc_feature (9)..(9): Xaa = Gly or Pro
  misc_feature (10)..(10): Xaa = Asp or Glu
  misc_feature (13)..(13): Xaa = Lys or Gln
  misc_feature (16)..(16): Xaa = Ala or Gly
  misc_feature (18)..(18): Xaa = Leu or Val
  misc_feature (20)..(20): Xaa = Leu or Met
  misc_feature (23)..(23): Xaa = Ala or Lys
  misc_feature (27)..(27): Xaa = Phe or Tyr
  misc_feature (29)..(29): Xaa = Phe or Leu
  misc_feature (30)..(30): Xaa = Ser or Thr
  misc_feature (31)..(31): Xaa = Asn or Arg
  misc_feature (33)..(33): Xaa = Gly  Ile or Val
  misc_feature (34)..(34): Xaa = Ile or Met
  misc_feature (35)..(35): Xaa = His  Asn or Ser
  misc_feature (38)..(38): Xaa = Lys or Arg
  misc_feature (40)..(40): Xaa = Lys or Thr
  misc_feature (42)..(42): Xaa = Asp or Gly
  misc_feature (43)..(43): Xaa = Lys or Gln
  misc_feature (44)..(44): Xaa = Gly or Arg
  misc_feature (48)..(48): Xaa = Ile or Val
  misc_feature (49)..(49): Xaa = Gly or Ser
  misc_feature (50)..(50): Xaa = Thr or Tyr
  misc_feature (52)..(52): Xaa = Ile or Asn
  misc_feature (53)..(53): Xaa = Pro or Ser
  misc_feature (54)..(54): Xaa = Gly or Tyr
  misc_feature (55)..(55): Xaa = Gly  Asn or Thr
  misc_feature (56)..(56): Xaa = Asp or Ile
  misc_feature (57)..(57): Xaa = Gly or Asn
  misc_feature (58)..(58): Xaa = Pro or Thr
  misc_feature (59)..(59): Xaa = Lys or Tyr
  misc_feature (61)..(61): Xaa = Asn or Ser
  misc_feature (62)..(62): Xaa = Asp or Glu
  misc_feature (63)..(63): Xaa = Lys  Arg or Ser
  misc_feature (64)..(64): Xaa = Phe or Val
  misc_feature (67)..(67): Xaa = Lys or Arg
  misc_feature (68)..(68): Xaa = Ala or Phe
  misc_feature (69)..(69): Xaa = Ser or Thr
  misc_feature (70)..(70): Xaa = Ile or Leu
  misc_feature (71)..(71): Xaa = Ser or Thr
  misc_feature (72)..(72): Xaa = Arg or Ser
  misc_feature (74)..(74): Xaa = Lys or Asn
  misc_feature (75)..(75): Xaa = Ala or Ser
  misc_feature (76)..(76): Xaa = Arg or Ser
  misc_feature (77)..(77): Xaa = Asn or Ser
  misc_feature (79)..(79): Xaa = Ala or Leu
  misc_feature (80)..(80): Xaa = Phe or Tyr
  misc_feature (81)..(81): Xaa = Leu or Met
  misc_feature (82)..(82): Xaa = Glu or Gln
  misc_feature (83)..(83): Xaa = Phe  Met or Val
  misc_feature (87)..(87): Xaa = Lys or Thr
  misc_feature (91)..(91): Xaa = Ser or Thr
  misc_feature (93)..(93): Xaa = Met or Val
  misc_feature (97)..(97): Xaa = Ala or Gly
  misc_feature (100)..(100): Xaa = Asn or Tyr
  misc_feature (101)..(101): Xaa = Arg or Tyr
  misc_feature (113)..(113): Xaa = Ala or Ser
EVQLXXSGXXLVXPGXSXKXSCXASGXTXXXYXXXWVXQXPXXXLEWXXXIXXXXXXXXYXXXXKGXXXXXXDXXXXTXXXXXSSLXSEDXAXYYCXRLXXGNAMDYWGQGTXVTVSS

SEQ ID NO: 79 - protein, 114 aa, Artificial Sequence
  5E6VL PRT 7E3 VL PRT 3A6 VL PRT 14E12 VL PRT 17B10 VL PRT
  misc_feature (12)..(12): Xaa = Ser or Thr
  misc_feature (14)..(14): Xaa = Ser or Thr
  misc_feature (15)..(15): Xaa = Ala or Val
  misc_feature (16)..(16): Xaa = Gly or Arg
  misc_feature (21)..(21): Xaa = Leu or Met
  misc_feature (22)..(22): Xaa = Asn or Ser
  misc_feature (32)..(32): Xaa = Asn or Ser
  misc_feature (40)..(40): Xaa = Ala or Thr
  misc_feature (56)..(56): Xaa = Gly or Trp
  misc_feature (76)..(76): Xaa = Asp or His
  misc_feature (78)..(78): Xaa = Ala or Thr
  misc_feature (97)..(97): Xaa = Asp or Val
  misc_feature (98)..(98): Xaa = Leu or Tyr
  misc_feature (99)..(99): Xaa = Ile  Ser or Tyr
  misc_feature (100)..(100): Xaa = Phe or Tyr
  misc_feature (102)..(102): Xaa = Phe or Leu
  misc_feature (106)..(106): Xaa = Ala or Ser
  misc_feature (111)..(111): Xaa = Asp or Glu
  misc_feature (112)..(112): Xaa = Ile or Leu
DIVMTQSPSSLXVXXXEKVTXXCKSSQSLLNXGNQKNYLXWYQQKPGQPPKLLIYXASTRESGVPDRFTGSGSGTXFXLTISSVQAEDLAVYYCQNXXXXPXTFGXGTKLXXKR

SEQ ID NO: 80 - protein, 32 aa, Artificial Sequence
  5E6H-FR3 7E3 H-FR3 14E12 H-FR3 17B10H-FR3
  misc_feature (1)..(1): Xaa = Lys or Arg
  misc_feature (14)..(14): Xaa = Phe or Tyr
  misc_feature (17)..(17): Xaa = Phe or Val
XATLTSDKSSSTAXMEXSSLTSEDSAVYYCAR

SEQ ID NO: 81 - protein, 448 aa, Artificial Sequence
  IMAB362 heavy chain
QVQLQQPGAELVRPGASVKLSCKASGYTFTSYWINWVKQRPGQGLEWIGNIYPSDSYTNYNQKFKDKATLTVDKSSSTAYMQLSSPTSEDSAVYYCTRSWRGNSFDYWGQGTTLTVSSASTKGPSVFPLAPSSKSTSGGTAALGCLVKDYFPEPVTVSWNSGALTSGVHTFPAVLQSSGLYSLSSVVTVPSSSLGTQTYICNVNHKPSNTKVDKRVEPKSCDKTHTCPPCPAPELLGGPSVFLFPPKPKDTLMISRTPEVTCVVVDVSHEDPEVKFNWYVDGVEVHNAKTKPREEQYNSTYRVVSVLTVLHQDWLNGKEYKCKVSNKALPAPIEKTISKAKGQPREPQVYTLPPSREEMTKNQVSLTCLVKGFYPSDIAVEWESNGQPENNYKTTPPVLDSDGSFFLYSKLTVDKSRWQQGNVFSCSVMHEALHNHYTQKSLSLSPGK

SEQ ID NO: 82 - protein, 220 aa, Artificial Sequence
  IMAB362 lighr chain
DIVMTQSPSSLTVTAGEKVTMSCKSSQSLLNSGNQKNYLTWYQQKPGQPPKLLIYWASTRESGVPDRFTGSGSGTDFTLTISSVQAEDLAVYYCQNDYSYPFTFGSGTKLEIKRTVAAPSVFIFPPSDEQLKSGTASVVCLLNNFYPREAKVQWKVDNALQSGNSQESVTEQDSKDSTYSLSSTLTLSKADYEKHKVYACEVTHQGLSSPVTKSFNRGEC

SEQ ID NO: 83 - protein, 45 aa, Artificial Sequence
  human CD8 hinge region
TTTPAPRPPTPAPTIASQPLSLRPEACRPAAGGAVHTRGLDFACD

SEQ ID NO: 84 - protein, 24 aa, Artificial Sequence
  human CD8 transmembrane domain
IYIWAPLAGTCGVLLLSLVITLYC

SEQ ID NO: 85 - protein, 42 aa, Artificial Sequence
  human 4-1BB costimulatory domain
KRGRKKLLYIFKQPFMRPVQTTQEEDGCSCRFPEEEEGGCEL

SEQ ID NO: 86 - protein, 112 aa, Artificial Sequence
  CD3   intracellular signaling domain
RVKFSRSADAPAYQQGQNQLYNELNLGRREEYDVLDKRRGRDPEMGGKPRRKNPQEGLYNELQKDKMAEAYSEIGMKGERRRGKGHDGLYQGLSTATKDTYDALHMQALPPR

SEQ ID NO: 87 - protein, 18 aa, Artificial Sequence
  T2A self-cutting peptide
EGRGSLLTCGDVEENPGP

SEQ ID NO: 88 - protein, 21 aa, Artificial Sequence
  human CD8 signal pepetide
MALPVTALLLPLALLLHAARP

SEQ ID NO: 89 - protein, 18 aa, Artificial Sequence
  single-chain antibody linker
ASTGGGGSGGGGSGGGGS

SEQ ID NO: 90 - protein, 250 aa, Artificial Sequence
  5E6 scFv
QVQLVQSGAEVKKPGASVKVSCKASGYTFTNYVMNWVRQAPGQRLEWMGYINPYNDGTKYNERFKGRVTITRDTSASTAYMELSSLRSEDTAVYYCARLYRGNAMDYWGQGTLVTVSSASTGGGGSGGGGSGGGGSDIVMTQSPDSLAVSLGERATINCKSSQSLLASGNQKNYLTWYQQKPGQPPKLLIYWASTRESGVPDRFSGSGSGTDFTLTISSLQAEDVAVYYCQNVYIYPFTFGQGTKLEIKR

SEQ ID NO: 91 - protein, 416 aa, Artificial Sequence
  Ori
EGRGSLLTCGDVEENPGPMGAVLRSLLACSFCVLLRAEQKLISEEDLEPPTCSPQQFTCFTGEIDCIPVAWRCDGFTECEDHSDELNCPVCSESQFQCASGQCIDGALRCNGDANCQDKSDEKNCEVLCLIDQFRCANGQCIGKHKKCDHNVDCSDKSDELDCYPTEEPAPQATNTVGSVIGVIVTIFVSGTVYFICQRMLCPRMKGDGETMTNDYVVHGPASVPLGYVPHPSSLSGSLPGMSRGKSMISSLSIMGGSSGPPYDRAHVTGASSSSSSSTKGTYFPAILNPPPSPATERSHYTMEFGYSSNSPSTHRSYSYRPYSYRHFAPPTTPCSTDVCDSDYAPSRRMTSVATAKGYTSDLNYDSEPVPPPPTPRSQYLSAEENYESCPPSPYTERSYSHHLYPPPPSPCTDSS

SEQ ID NO: 92 - protein, 118 aa, Artificial Sequence
  Standard scFv VH
QVQLQESGPGLIKPSQTLSLTCTVSGGSISSGYNWHWIRQPPGKGLEWIGYIHYTGSTNYNPALRSRVTISVDTSKNQFSLKLSSVTAADTAIYYCARIYNGNSFPYWGQGTTVTVSS

SEQ ID NO: 93 - protein, 114 aa, Artificial Sequence
  Standard scFv VL
DIVMTQSPDSLAVSLGERATINCKSSQSLFNSGNQKNYLTWYQQKPGQPPKLLIYWASTRESGVPDRFSGSGSGTDFTLTISSLQAEDVAVYYCQNAYSFPYTFGGGTKLEIKR